European Patent Application EP 4 509 526 A2, published February 19, 2025. Title: 抗甲状腺球蛋白抗体、试剂盒和用途. Applicant: 深圳迈瑞生物医疗电子股份有限公司. Application CN. The sequence listing filed with the application follows.

SEQUENCE LISTING (72 sequences)

SEQ ID NO: 1 - protein, 5 aa, synthetic construct
  source 1..5: note = H-CDR1 amino acid sequence of TG01
NYGMN

SEQ ID NO: 2 - protein, 17 aa, synthetic construct
  source 1..17: note = H-CDR2 amino acid sequence of TG01
WINTYTGEPTYADDFKG

SEQ ID NO: 3 - protein, 10 aa, synthetic construct
  source 1..10: note = H-CDR3 amino acid sequence of TG01
RRETARALDS

SEQ ID NO: 4 - protein, 16 aa, synthetic construct
  source 1..16: note = L-CDR1 amino acid sequence of TG01
CRSSQSLVHSNGDTYL

SEQ ID NO: 5 - protein, 7 aa, synthetic construct
  source 1..7: note = L-CDR2 amino acid sequence of TG01
YKVSNRF

SEQ ID NO: 6 - protein, 10 aa, synthetic construct
  source 1..10: note = L-CDR3 amino acid sequence of TG01
CSQSTHVPFT

SEQ ID NO: 7 - protein, 5 aa, synthetic construct
  source 1..5: note = H-CDR1 amino acid sequence of TG02/hTG02
DYDMA

SEQ ID NO: 8 - protein, 17 aa, synthetic construct
  source 1..17: note = H-CDR2 amino acid sequence of TG02/hTG02
SISFSRGRTYYRDSVKG

SEQ ID NO: 9 - protein, 10 aa, synthetic construct
  source 1..10: note = H-CDR3 amino acid sequence of TG02/hTG02
QGRYSSFIDA

SEQ ID NO: 10 - protein, 16 aa, synthetic construct
  source 1..16: note = L-CDR1 amino acid sequence of TG02/hTG02
RSSQSLVHSDGNTYLH

SEQ ID NO: 11 - protein, 7 aa, synthetic construct
  source 1..7: note = L-CDR2 amino acid sequence of TG02/hTG02
RVSNRFS

SEQ ID NO: 12 - protein, 9 aa, synthetic construct
  source 1..9: note = L-CDR3 amino acid sequence of TG02/hTG02
LQSTHFPPT

SEQ ID NO: 13 - protein, 5 aa, synthetic construct
  source 1..5: note = H-CDR1 amino acid sequence of TG03/hTG03
QYDMA

SEQ ID NO: 14 - protein, 17 aa, synthetic construct
  source 1..17: note = H-CDR2 amino acid sequence of TG03/hTG03
SISPFGPRTYYRDSVKG

SEQ ID NO: 15 - protein, 10 aa, synthetic construct
  source 1..10: note = H-CDR3 amino acid sequence of TG03/hTG03
QGRYSSFMDA

SEQ ID NO: 16 - protein, 16 aa, synthetic construct
  source 1..16: note = L-CDR1 amino acid sequence of TG03/hTG03
RSSQSLVHSDGNTYLH

SEQ ID NO: 17 - protein, 7 aa, synthetic construct
  source 1..7: note = L-CDR2 amino acid sequence of TG03/hTG03
RVSTRFS

SEQ ID NO: 18 - protein, 9 aa, synthetic construct
  source 1..9: note = L-CDR3 amino acid sequence of TG03/hTG03
LQSTHFPPT

SEQ ID NO: 19 - protein, 5 aa, synthetic construct
  source 1..5: note = H-CDR1 amino acid sequence of TG04/hTG04
HHDMA

SEQ ID NO: 20 - protein, 17 aa, synthetic construct
  source 1..17: note = H-CDR2 amino acid sequence of TG04/hTG04
SISFSYGRTYYRDSVKV

SEQ ID NO: 21 - protein, 10 aa, synthetic construct
  source 1..10: note = H-CDR3 amino acid sequence of TG04/hTG04
QGRYNSFMDA

SEQ ID NO: 22 - protein, 16 aa, synthetic construct
  source 1..16: note = L-CDR1 amino acid sequence of TG04/hTG04
RSSQSLVHSDGNTHLH

SEQ ID NO: 23 - protein, 7 aa, synthetic construct
  source 1..7: note = L-CDR2 amino acid sequence of TG04/hTG04
RVSNRFS

SEQ ID NO: 24 - protein, 9 aa, synthetic construct
  source 1..9: note = L-CDR3 amino acid sequence of TG04/hTG04
LQSTHFPPT

SEQ ID NO: 25 - protein, 5 aa, synthetic construct
  source 1..5: note = H-CDR1 amino acid sequence of TG05/hTG05
NYDLA

SEQ ID NO: 26 - protein, 17 aa, synthetic construct
  source 1..17: note = H-CDR2 amino acid sequence of TG05/hTG05
SISRSRGDTYYRDSVKG

SEQ ID NO: 27 - protein, 10 aa, synthetic construct
  source 1..10: note = H-CDR3 amino acid sequence of TG05/hTG05
QDYYSSFLDY

SEQ ID NO: 28 - protein, 16 aa, synthetic construct
  source 1..16: note = L-CDR1 amino acid sequence of TG05/hTG05
RSSQSLVHSDGKTYLH

SEQ ID NO: 29 - protein, 7 aa, synthetic construct
  source 1..7: note = L-CDR2 amino acid sequence of TG05/hTG05
RVSNRFS

SEQ ID NO: 30 - protein, 9 aa, synthetic construct
  source 1..9: note = L-CDR3 amino acid sequence of TG05/hTG05
LQSTHFPPT

SEQ ID NO: 31 - protein, 5 aa, synthetic construct
  source 1..5: note = H-CDR1 amino acid sequence of TG06/hTG06
NYGMA

SEQ ID NO: 32 - protein, 17 aa, synthetic construct
  source 1..17: note = H-CDR2 amino acid sequence of TG06/hTG06
SITYDGTRTYSRDSVKG

SEQ ID NO: 33 - protein, 7 aa, synthetic construct
  source 1..7: note = H-CDR3 amino acid sequence of TG06/hTG06
HPGSFDY

SEQ ID NO: 34 - protein, 16 aa, synthetic construct
  source 1..16: note = L-CDR1 amino acid sequence of TG06/hTG06
RSSQSLLHSNGNTYLE

SEQ ID NO: 35 - protein, 7 aa, synthetic construct
  source 1..7: note = L-CDR2 amino acid sequence of TG06/hTG06
KVSNRVS

SEQ ID NO: 36 - protein, 9 aa, synthetic construct
  source 1..9: note = L-CDR3 amino acid sequence of TG06/hTG06
FQATHDPVT

SEQ ID NO: 37 - DNA, 15 bp, synthetic construct
  source 1..15: mol_type = other DNA; note = H-CDR1 nucleotide sequence of TG01
aactatggaatgaac

SEQ ID NO: 38 - DNA, 51 bp, synthetic construct
  source 1..51: mol_type = other DNA; note = H-CDR2 nucleotide sequence of TG01
tggataaacacctacactggagagccaacatatgctgatgacttcaaggga

SEQ ID NO: 39 - DNA, 30 bp, synthetic construct
  source 1..30: mol_type = other DNA; note = H-CDR3 nucleotide sequence of TG01
agaagagagacagctcgggctcttgactcc

SEQ ID NO: 40 - DNA, 48 bp, synthetic construct
  source 1..48: mol_type = other DNA; note = L-CDR1 nucleotide sequence of TG01
tgcagatctagtcagagccttgtacacagtaatggagacacctattta

SEQ ID NO: 41 - DNA, 21 bp, synthetic construct
  source 1..21: mol_type = other DNA; note = L-CDR2 nucleotide sequence of TG01
tacaaagtttccaaccgattt

SEQ ID NO: 42 - DNA, 30 bp, synthetic construct
  source 1..30: mol_type = other DNA; note = L-CDR3 nucleotide sequence of TG01
tgctctcaaagtacacatgttccattcacg

SEQ ID NO: 43 - DNA, 15 bp, synthetic construct
  source 1..15: mol_type = other DNA; note = H-CDR1 nucleotide sequence of TG02/hTG02
gactatgacatggcc

SEQ ID NO: 44 - DNA, 51 bp, synthetic construct
  source 1..51: mol_type = other DNA; note = H-CDR2 nucleotide sequence of TG02/hTG02
tccattagttttagtcgtggtcgcacttattatcgagactccgtgaagggc

SEQ ID NO: 45 - DNA, 30 bp, synthetic construct
  source 1..30: mol_type = other DNA; note = H-CDR3 nucleotide sequence of TG02/hTG02
cagggacgatacagctcctttatcgatgcc

SEQ ID NO: 46 - DNA, 48 bp, synthetic construct
  source 1..48: mol_type = other DNA; note = L-CDR1 nucleotide sequence of TG02/hTG02
cggtcaagtcagagccttgtacacagtgatggaaacacctacttgcat

SEQ ID NO: 47 - DNA, 21 bp, synthetic construct
  source 1..21: mol_type = other DNA; note = L-CDR2 nucleotide sequence of TG02/hTG02
cgggtttccaacagattttct

SEQ ID NO: 48 - DNA, 27 bp, synthetic construct
  source 1..27: mol_type = other DNA; note = L-CDR3 nucleotide sequence of TG02/hTG02
ttacaaagtacacattttcctccgacg

SEQ ID NO: 49 - DNA, 15 bp, synthetic construct
  source 1..15: mol_type = other DNA; note = H-CDR1 nucleotide sequence of TG03/hTG03
cagtatgacatggcc

SEQ ID NO: 50 - DNA, 51 bp, synthetic construct
  source 1..51: mol_type = other DNA; note = H-CDR2 nucleotide sequence of TG03/hTG03
tccattagtccttttggtcctagaacttattatcgagactccgtgaagggc

SEQ ID NO: 51 - DNA, 30 bp, synthetic construct
  source 1..30: mol_type = other DNA; note = H-CDR3 nucleotide sequence of TG03/hTG03
cagggacggtactcctcctttatggatgcc

SEQ ID NO: 52 - DNA, 48 bp, synthetic construct
  source 1..48: mol_type = other DNA; note = L-CDR1 nucleotide sequence of TG03/hTG03
cggtcaagtcagagccttgtacacagtgatggaaacacctacttacat

SEQ ID NO: 53 - DNA, 21 bp, synthetic construct
  source 1..21: mol_type = other DNA; note = L-CDR2 nucleotide sequence of TG03/hTG03
cgggtttccaccagattttct

SEQ ID NO: 54 - DNA, 27 bp, synthetic construct
  source 1..27: mol_type = other DNA; note = L-CDR3 nucleotide sequence of TG03/hTG03
ttacaaagtacacattttcctccgacg

SEQ ID NO: 55 - DNA, 15 bp, synthetic construct
  source 1..15: mol_type = other DNA; note = H-CDR1 nucleotide sequence of TG04/hTG04
caccatgacatggcc

SEQ ID NO: 56 - DNA, 51 bp, synthetic construct
  source 1..51: mol_type = other DNA; note = H-CDR2 nucleotide sequence of TG04/hTG04
tccattagttttagttatggtcgcacttattatcgagactccgtgaaggtc

SEQ ID NO: 57 - DNA, 30 bp, synthetic construct
  source 1..30: mol_type = other DNA; note = H-CDR3 nucleotide sequence of TG04/hTG04
cagggacgatacaactcctttatggatgcc

SEQ ID NO: 58 - DNA, 48 bp, synthetic construct
  source 1..48: mol_type = other DNA; note = L-CDR1 nucleotide sequence of TG04/hTG04
cggtcaagtcagagccttgttcacagtgatggaaatacccacttgcat

SEQ ID NO: 59 - DNA, 21 bp, synthetic construct
  source 1..21: mol_type = other DNA; note = L-CDR2 nucleotide sequence of TG04/hTG04
cgggtgtccaacagattctct

SEQ ID NO: 60 - DNA, 27 bp, synthetic construct
  source 1..27: mol_type = other DNA; note = L-CDR3 nucleotide sequence of TG04/hTG04
ttacaaagtacacattttcctccgacg

SEQ ID NO: 61 - DNA, 15 bp, synthetic construct
  source 1..15: mol_type = other DNA; note = H-CDR1 nucleotide sequence of TG05/hTG05
aactatgacctggcc

SEQ ID NO: 62 - DNA, 51 bp, synthetic construct
  source 1..51: mol_type = other DNA; note = H-CDR2 nucleotide sequence of TG05/hTG05
tccattagtcgtagtcgtggtgacacttactatcgagactccgtaaagggc

SEQ ID NO: 63 - DNA, 30 bp, synthetic construct
  source 1..30: mol_type = other DNA; note = H-CDR3 nucleotide sequence of TG05/hTG05
caagattactatagcagcttccttgattac

SEQ ID NO: 64 - DNA, 48 bp, synthetic construct
  source 1..48: mol_type = other DNA; note = L-CDR1 nucleotide sequence of TG05/hTG05
cggtcaagtcagagcctggtacacagtgatggaaaaacctacttacat

SEQ ID NO: 65 - DNA, 21 bp, synthetic construct
  source 1..21: mol_type = other DNA; note = L-CDR2 nucleotide sequence of TG05/hTG05
cgggtttccaacagattttct

SEQ ID NO: 66 - DNA, 27 bp, synthetic construct
  source 1..27: mol_type = other DNA; note = L-CDR3 nucleotide sequence of TG05/hTG05
ttgcaaagtacacattttcctccgacg

SEQ ID NO: 67 - DNA, 15 bp, synthetic construct
  source 1..15: mol_type = other DNA; note = H-CDR1 nucleotide sequence of TG06/hTG06
aattatggcatggcc

SEQ ID NO: 68 - DNA, 51 bp, synthetic construct
  source 1..51: mol_type = other DNA; note = H-CDR2 nucleotide sequence of TG06/hTG06
tccattacttatgatggtactagaacttactctcgagactccgtgaagggc

SEQ ID NO: 69 - DNA, 21 bp, synthetic construct
  source 1..21: mol_type = other DNA; note = H-CDR3 nucleotide sequence of TG06/hTG06
caccccgggtcctttgattac

SEQ ID NO: 70 - DNA, 48 bp, synthetic construct
  source 1..48: mol_type = other DNA; note = L-CDR1 nucleotide sequence of TG06/hTG06
aggtctagtcagagcctgctacatagtaatggaaacacttatttggaa

SEQ ID NO: 71 - DNA, 21 bp, synthetic construct
  source 1..21: mol_type = other DNA; note = L-CDR2 nucleotide sequence of TG06/hTG06
aaggtttccaaccgagtttct

SEQ ID NO: 72 - DNA, 27 bp, synthetic construct
  source 1..27: mol_type = other DNA; note = L-CDR3 nucleotide sequence of TG06/hTG06
ttccaagctacacatgatccggtcacg